European Patent Application EP 4 316 495 A1, published February 7, 2024. Title: Nucleic acid molecule conjugate with extended in vivo half-life. Applicant: APTACURE THERAPEUTICS LIMITED. The sequence listing filed with the application follows.

SEQUENCE LISTING (26 sequences)

SEQ ID NO: 1 - DNA, 40 bp, Artificial Sequence
  aptscl56
cggggtgtgggttcgtcgttagcttgatttggcagctgcc

SEQ ID NO: 2 - DNA, 42 bp, Artificial Sequence
  aptscl132
cccagacgagacacctcatgcttttccccgggggaggggtat

SEQ ID NO: 3 - DNA, 76 bp, Artificial Sequence
  aptscl6
cgtacggtcgacgctagctggaagggtgggggcggggggtcctcgcctcgaacgtacgcacgtggagctcggatcc

SEQ ID NO: 4 - DNA, 76 bp, Artificial Sequence
  aptscl9
cgtacggtcgacgctagctgggggtagggggaccctggctagttagtcaccgtttcgacacgtggagctcggatcc

SEQ ID NO: 5 - DNA, 76 bp, Artificial Sequence
  aptscl15
cgtacggtcgacgctagcgagggggccaactatgcttagtgggggggttgaccgtatccacgtggagctcggatcc

SEQ ID NO: 6 - DNA, 76 bp, Artificial Sequence
  aptscl46
cgtacggtcgacgctagcgggtggattaagggggccccgtctgtaggcgattggcgaacacgtggagctcggatcc

SEQ ID NO: 7 - DNA, 76 bp, Artificial Sequence
  aptscl51
cgtacggtcgacgctagctgggggtagggggtccttggctacggtgattcggatgtgacacgtggagctcggatcc

SEQ ID NO: 8 - DNA, 56 bp, Artificial Sequence
  aptscl1
cgtacggtcgacgctagctcttgttcatcgatcctacgcacgtggagctcggatcc

SEQ ID NO: 9 - DNA, 54 bp, Artificial Sequence
  aptscl2
cgtacggtcgacgctagccagccaaagacagagatgcacgtggagctcggatcc

SEQ ID NO: 10 - DNA, 55 bp, Artificial Sequence
  aptscl3
cgtacggtcgacgctagctgttgtacatcgccttacgcacgtggagctcggatcc

SEQ ID NO: 11 - DNA, 56 bp, Artificial Sequence
  aptscl5
cgtacggtcgacgctagctgttgttcatcgacttgacgcacgtggagctcggatcc

SEQ ID NO: 12 - DNA, 51 bp, Artificial Sequence
  aptscl8
cgtacggtcgacgctagccggcgaaattgctaccacgtggagctcggatcc

SEQ ID NO: 13 - DNA, 52 bp, Artificial Sequence
  aptscl12
cgtacggtcgacgctagccgttgactcgttgctacacgtggagctcggatcc

SEQ ID NO: 14 - DNA, 55 bp, Artificial Sequence
  aptscl16
cgtacggtcgacgctagctggtttcatcgatcgtatccacgtggagctcggatcc

SEQ ID NO: 15 - DNA, 55 bp, Artificial Sequence
  aptscl22
cgtacggtcgacgctagctgggtttatcgactagttccacgtggagctcggatcc

SEQ ID NO: 16 - DNA, 51 bp, Artificial Sequence
  aptscl29
cgtacggtcgacgctagccggagacctgaggttcacgtggagctcggatcc

SEQ ID NO: 17 - DNA, 56 bp, Artificial Sequence
  aptscl32
cgtacggtcgacgctagctgtgttaatcgccgtacctccacgtggagctcggatcc

SEQ ID NO: 18 - protein, 190 aa, Homo sapiens
QGWQAFKNDATEIIPELGEYPEPPPELENNKTMNRAENGGRPPHHPFETKDVSEYSCRELHFTRYVTDGPCRSAKPVTELVCSGQCGPARLLPNAIGRGKWWRPSGPDFRCIPDRYRAQRVQLLCPGGEAPRARKVRLVASCKCKRLTRFHNQSELKDFGTEAARPQKGRKPRPRARSAKANQAELENAY

SEQ ID NO: 19 - DNA, 49 bp, Artificial Sequence
  aptscl3-1
gtcgacgctagctgttgtacatcgccttacgcacgtggagctcggatcc

SEQ ID NO: 20 - DNA, 49 bp, Artificial Sequence
  aptscl3-2
cgtacggtcgacgctagctgttgtacatcgccttacgcacgtggagctc

SEQ ID NO: 21 - DNA, 37 bp, Artificial Sequence
  aptscl3-3
gctagctgttgtacatcgccttacgcacgtggagctc

SEQ ID NO: 22 - DNA, 37 bp, Artificial Sequence
  aptscl3-4
gtcgacgctagctgttgtacatcgccttacgcacgtg

SEQ ID NO: 23 - DNA, 31 bp, Artificial Sequence
  aptscl3-5
gctagctgttgtacatcgccttacgcacgtg

SEQ ID NO: 24 - DNA, 25 bp, Artificial Sequence
  aptscl3-6
tgttgtacatcgccttacgcacgtg

SEQ ID NO: 25 - DNA, 40 bp, Artificial Sequence
  modified aptscl56
cggggtgtgggttcgtcgttagcttgatttggcagcugcc

SEQ ID NO: 26 - DNA, 38 bp, Artificial Sequence
  APTDKK1
cgtacggtcgacgctagctggtggttggggtgggtggt